European Patent Application EP 4 501 357 A1, published February 5, 2025. Title: Pharmaceutical composition for prevention, suppression or treatment of symptoms associated with pseudo-allergic reaction. Applicant: 学校法人　高崎健康福祉大学. The sequence listing filed with the application follows.

SEQUENCE LISTING (35 sequences)

SEQ ID NO: 1 - protein, 330 aa, Homo sapiens
MDPTTPAWGTESTTVNGNDQALLLLCGKETLIPVFLILFIALVGLVGNGFVLWLLGFRMRRNAFSVYVLSLAGADFLFLCFQIINCLVYLSNFFCSISINFPSFFTTVMTCAYLAGLSMLSTVSTERCLSVLWPIWYRCRRPRHLSAVVCVLLWALSLLLSILEGKFCGFLFSDGDSGWCQTFDFITAAWLIFLFMVLCGSSLALLVRILCGSRGLPLTRLYLTILLTVLVFLLCGLPFGIQWFLILWIWKDSDVLFCHIHPVSVVLSSLNSSANPIIYFFVGSFRKQWRLQQPILKLALQRALQDIAEVDHSEGCFRQGTPEMSRSSLV

SEQ ID NO: 2 - DNA, 2440 bp, Homo sapiens
  source 1..2440: mol_type = other DNA
tggctacaggaaagggccaccaggcagggctatgtccttaggtagaaaaacactgccactgccaactcacagcccttcagggcgcagggagagagccaggaaatttttaaaaaatcatcccccaatctactgtcaatgtgtccctttggctgaaaaaaaaagtcaccctccaatctcctgtcaatgtgtaccctttggagcctgagtgaaagacagcccattgacgaggcacagacatgtctcctcccaggatgcaaagtgtcacttctttggactagtctctcactatcatcataaatgccttgagaatggaatgtggttgggaaaaaaagggattgggagtacataggtactcccagctataagtacacaggggcaccagtggaggttttctgagcatggatccaaccaccccggcctggggaacagaaagtacaacagtgaatggaaatgaccaagcccttcttctgctttgtggcaaggagaccctgatcccggtcttcctgatccttttcattgccctggtcgggctggtaggaaacgggtttgtgctctggctcctgggcttccgcatgcgcaggaacgccttctctgtctacgtcctcagcctggccggggccgacttcctcttcctctgcttccagattataaattgcctggtgtacctcagtaacttcttctgttccatctccatcaatttccctagcttcttcaccactgtgatgacctgtgcctaccttgcaggcctgagcatgctgagcaccgtcagcaccgagcgctgcctgtccgtcctgtggcccatctggtatcgctgccgccgccccagacacctgtcagcggtcgtgtgtgtcctgctctgggccctgtccctactgctgagcatcttggaagggaagttctgtggcttcttatttagtgatggtgactctggttggtgtcagacatttgatttcatcactgcagcgtggctgatttttttattcatggttctctgtgggtccagtctggccctgctggtcaggatcctctgtggctccaggggtctgccactgaccaggctgtacctgaccatcctgctcacagtgctggtgttcctcctctgcggcctgccctttggcattcagtggttcctaatattatggatctggaaggattctgatgtcttattttgtcatattcatccagtttcagttgtcctgtcatctcttaacagcagtgccaaccccatcatttacttcttcgtgggctcttttaggaagcagtggcggctgcagcagccgatcctcaagctggctctccagagggctctgcaggacattgctgaggtggatcacagtgaaggatgcttccgtcagggcaccccggagatgtcgagaagcagtctggtgtagagatggacagcctctacttccatcagatatatgtggctttgagaggcaactttgcccctgtctgtctgatttgctgaactttctcagtcctgattttaaaacagttaagagagtccttgtgaggattaagtgagacagtgcctatgaaacaaacactaagtgcagtgtctctggaactgccttactcacaggcttccaccacagccctatgagagctttgccaactctgcggtccatgactgttcccacttttaatgaatcctacctttcgcagaaggctgaaagcagggcagaaaagatctacatttctttggacactgcacttgatagggactcaaagaatgttatatttttaattaatttctttttctcttccgtacaatttctgtctcaacaaaattagaagaattaaatttaaaactagctccaaaagagcagtcgtctttcattttggcagaccttagaatatccccctagcttaataaatctttgttgaatggcttaatgaatgaataaactggttaatgtttaagttaaacctctgaaaagtctccatttaccagatttgagtcactaaatttattgctttcactacttttgaattttgcaaacatgaaattaagttttataattagataaatcaatgtcaacacatatttaaagtttgaggtacactgtcttcctgtggtttcctttcacatgccatcccttaaaatcccagctacacgccttcccattccttcccctttgcctttgttctaatcttccctctctgggggctctctaattcgtcctggaagtttccagtggtcttatagactccatgttcttggaggacaggctgtatgtcagatttaccttttattccgaagaactcggagcatttattttgttaattaaattgcacatatttttaaaagttacgtgttccacagaataaaatactaattgtaaaaaaaaaaaaaaaaaaaaaaaaaaaaaaaaaaaaaaaaaaaaaaaaaaaaaaaaaaaaaaaaaaaaaaaaaaaaaaaaaaaaaaaaaaaaaaaaa

SEQ ID NO: 3 - DNA, 1997 bp, Homo sapiens
  source 1..1997: mol_type = other DNA
cgcagcgagcctgccggagctggtgggtggagctacgaccgggagccgacggtggcgaggggacccacagtgtccaaggcgcggagcggtcggcggagccatggcgggctgctgctccgtgctcgggtccttcctgttcgagtacgacacgccgcgcatcgtgctcatccgcagccgtaaagtggggctcatgaaccgcgcggtgcagctgctcatcctggcttacgtcatcgggtgggtgttcgtgtgggaaaagggctaccaggaaacggactccgtggtcagctcggtgacaaccaaagccaaaggtgtggctgtgaccaacacctctcagcttggattccggatctgggacgtggcggactatgtgattccagctcaggaggaaaactccctcttcatcatgaccaacatgatcgtcaccgtgaaccagacacagagcacctgtccagagattcctgataagaccagcatttgtaattcagacgccgactgcactcctggctccgtggacacccacagcagtggagttgcgactggaagatgtgttcctttcaatgagtctgtgaagacctgtgaggtggctgcatggtgcccggtggagaacgacgttggcgtgccaacgccggctttcttaaaggctgcagaaaacttcaccctcttggtaaagaacaacatctggtaccccaagtttaacttcagcaagaggaacatcctccccaacatcaccacgtcctacctcaaatcgtgcatttacaatgctcaaacggatcccttctgccccatattccgtcttggcacaatcgtgggggacgcgggacatagcttccaggagatggcagttgagggaggcatcatgggtatccagatcaagtgggactgcaacctggatagagccgcctccctttgcctgcccagatattccttccggcgcctggacacccgggacctggaacacaatgtgtctcctggctacaatttcaggtttgccaagtactacagggacctggccggcaaagagcagcgcacactcaccaaggcgtacggcatccgctttgacatcatcgtgtttggaaaggctgggaagtttgacatcatccctaccatgatcaacgttggctctggcttggcgctcctcggggtggcgacggtgctctgtgacgtcatagtcctctactgcatgaagaagaaatactactaccgggacaagaaatataagtatgtggaagactacgagcagggtctttcgggggagatgaaccagtgacgcctaaagttacatttccaccccgctcagcccgcgaagcagaaagatggggagagatggctactgcgtctgtcactctagagaaagctccagagtttcagctcagttctccactccacaaatactcagggttgccaagcacatcttgttggagcccggctcttgctctgctgctcagatgggcttccagatacaagaatcctcctgcttctgcctctaggaatgctgggatcaaacatgtcacttgcaatgcccatttcccatggggagtttggcattttttacattttaccctttccttttgtatacatctaaggctgccctcagacgcaagacgttcttccaccctatacacccttttaatctcactgtgtgtgggaggggggtcgtttgcacacgacgcacggtggatgtctggtgtgctgttggctgggccacctgtggcttatacagtgtgagcgtatggaggtaggaagggtctgagagcagagacactgctgtggcttacggacaggcccaggctctgtccacgcactttatttctaaggaaggaggctctctcaggtgctgtcagcaggcctgggacaccattcctcttccctataatcagagaagttgtccttgtagcaaaggcagggttagcttttccttttataagggctgtgttgaaatgacctaggaccaaacattaaaagaaataattttttaaaaaaaaaaaaaaaaaaaaaaa

SEQ ID NO: 4 - DNA, 20 bp, synthetic construct
  misc_feature 1..20: note = Synthetic primer
  source 1..20: mol_type = other DNA
gaaggtggcatatgccaaga

SEQ ID NO: 5 - DNA, 20 bp, synthetic construct
  misc_feature 1..20: note = Synthetic primer
  source 1..20: mol_type = other DNA
tgtcatccacctctacagga

SEQ ID NO: 6 - DNA, 20 bp, synthetic construct
  misc_feature 1..20: note = Synthetic primer
  source 1..20: mol_type = other DNA
acttcgtgtggtacgtcttc

SEQ ID NO: 7 - DNA, 20 bp, synthetic construct
  misc_feature 1..20: note = Synthetic primer
  source 1..20: mol_type = other DNA
tgatccccttgactttggtg

SEQ ID NO: 8 - DNA, 22 bp, synthetic construct
  misc_feature 1..22: note = Synthetic primer
  source 1..22: mol_type = other DNA
ggattctgtccagagaatgagg

SEQ ID NO: 9 - DNA, 20 bp, synthetic construct
  misc_feature 1..20: note = Synthetic primer
  source 1..20: mol_type = other DNA
ggcttccatcatgataggca

SEQ ID NO: 10 - DNA, 20 bp, synthetic construct
  misc_feature 1..20: note = Synthetic primer
  source 1..20: mol_type = other DNA
aacatgatcgtcaccgtgaa

SEQ ID NO: 11 - DNA, 20 bp, synthetic construct
  misc_feature 1..20: note = Synthetic primer
  source 1..20: mol_type = other DNA
aatggaacacaccttccagt

SEQ ID NO: 12 - DNA, 20 bp, synthetic construct
  misc_feature 1..20: note = Synthetic primer
  source 1..20: mol_type = other DNA
gaaaactggtcgctgtctac

SEQ ID NO: 13 - DNA, 20 bp, synthetic construct
  misc_feature 1..20: note = Synthetic primer
  source 1..20: mol_type = other DNA
gtagagattggtggagctga

SEQ ID NO: 14 - DNA, 18 bp, synthetic construct
  misc_feature 1..18: note = Synthetic primer
  source 1..18: mol_type = other DNA
ttgcaacctggacacgaa

SEQ ID NO: 15 - DNA, 18 bp, synthetic construct
  misc_feature 1..18: note = Synthetic primer
  source 1..18: mol_type = other DNA
tttctgctgcagctggaa

SEQ ID NO: 16 - DNA, 20 bp, synthetic construct
  misc_feature 1..20: note = Synthetic primer
  source 1..20: mol_type = other DNA
taagctgtaccagcggaaag

SEQ ID NO: 17 - DNA, 20 bp, synthetic construct
  misc_feature 1..20: note = Synthetic primer
  source 1..20: mol_type = other DNA
tgcaaagggaaggtgtagtc

SEQ ID NO: 18 - DNA, 20 bp, synthetic construct
  misc_feature 1..20: note = Synthetic primer
  source 1..20: mol_type = other DNA
cagaccccagaaatgtgtga

SEQ ID NO: 19 - DNA, 20 bp, synthetic construct
  misc_feature 1..20: note = Synthetic primer
  source 1..20: mol_type = other DNA
ctcgtgtctccattctgctt

SEQ ID NO: 20 - DNA, 22 bp, synthetic construct
  misc_feature 1..22: note = Synthetic primer
  source 1..22: mol_type = other DNA
gcctgtgcatatgtgagtgaag

SEQ ID NO: 21 - DNA, 22 bp, synthetic construct
  misc_feature 1..22: note = Synthetic primer
  source 1..22: mol_type = other DNA
cacgtacttgaagtcctcgttg

SEQ ID NO: 22 - DNA, 20 bp, synthetic construct
  misc_feature 1..20: note = Synthetic primer
  source 1..20: mol_type = other DNA
gtcttctctgcctaggtgtt

SEQ ID NO: 23 - DNA, 20 bp, synthetic construct
  misc_feature 1..20: note = Synthetic primer
  source 1..20: mol_type = other DNA
ccagagtgatcaagaaggga

SEQ ID NO: 24 - DNA, 18 bp, synthetic construct
  misc_feature 1..18: note = Synthetic primer
  source 1..18: mol_type = other DNA
tgcctttccacatcacca

SEQ ID NO: 25 - DNA, 20 bp, synthetic construct
  misc_feature 1..20: note = Synthetic primer
  source 1..20: mol_type = other DNA
gagcctctgtaagagatcgt

SEQ ID NO: 26 - DNA, 20 bp, synthetic construct
  misc_feature 1..20: note = Synthetic primer
  source 1..20: mol_type = other DNA
tcagccaataccaccttctc

SEQ ID NO: 27 - DNA, 18 bp, synthetic construct
  misc_feature 1..18: note = Synthetic primer
  source 1..18: mol_type = other DNA
tcctcattgccaagctgt

SEQ ID NO: 28 - DNA, 20 bp, synthetic construct
  misc_feature 1..20: note = Synthetic primer
  source 1..20: mol_type = other DNA
ccatgtgtgagatggggaaa

SEQ ID NO: 29 - DNA, 20 bp, synthetic construct
  misc_feature 1..20: note = Synthetic primer
  source 1..20: mol_type = other DNA
gctagggtgatgttgtctgt

SEQ ID NO: 30 - DNA, 20 bp, synthetic construct
  misc_feature 1..20: note = Synthetic primer
  source 1..20: mol_type = other DNA
tccagccgcaatatcttcag

SEQ ID NO: 31 - DNA, 20 bp, synthetic construct
  misc_feature 1..20: note = Synthetic primer
  source 1..20: mol_type = other DNA
ataatggggtccagacacac

SEQ ID NO: 32 - DNA, 20 bp, synthetic construct
  misc_feature 1..20: note = Synthetic primer
  source 1..20: mol_type = other DNA
acgtccaagacacacatcag

SEQ ID NO: 33 - DNA, 20 bp, synthetic construct
  misc_feature 1..20: note = Synthetic primer
  source 1..20: mol_type = other DNA
tagacccacagagaacacca

SEQ ID NO: 34 - DNA, 20 bp, synthetic construct
  misc_feature 1..20: note = Synthetic primer
  source 1..20: mol_type = other DNA
tgctgagtatgtcgtggagt

SEQ ID NO: 35 - DNA, 20 bp, synthetic construct
  misc_feature 1..20: note = Synthetic primer
  source 1..20: mol_type = other DNA
catacttggcaggtttctcc